European Patent Application EP 4 122 487 A1, published January 25, 2023. Title: Factor VIII POLYPEPTIDE FORMULATIONS. Applicant: Bioverativ Therapeutics Inc. The sequence listing filed with the application follows.

SEQUENCE LISTING (18 sequences)

SEQ ID NO: 1 - DNA, 5052 bp, Artificial Sequence
  B-Domain Deleted FVIIIFc
atgcaaatagagctctccacctgcttctttctgtgccttttgcgattctgctttagtgccaccagaagatactacctgggtgcagtggaactgtcatgggactatatgcaaagtgatctcggtgagctgcctgtggacgcaagatttcctcctagagtgccaaaatcttttccattcaacacctcagtcgtgtacaaaaagactctgtttgtagaattcacggatcaccttttcaacatcgctaagccaaggccaccctggatgggtctgctaggtcctaccatccaggctgaggtttatgatacagtggtcattacacttaagaacatggcttcccatcctgtcagtcttcatgctgttggtgtatcctactggaaagcttctgagggagctgaatatgatgatcagaccagtcaaagggagaaagaagatgataaagtcttccctggtggaagccatacatatgtctggcaggtcctgaaagagaatggtccaatggcctctgacccactgtgccttacctactcatatctttctcatgtggacctggtaaaagacttgaattcaggcctcattggagccctactagtatgtagagaagggagtctggccaaggaaaagacacagaccttgcacaaatttatactactttttgctgtatttgatgaagggaaaagttggcactcagaaacaaagaactccttgatgcaggatagggatgctgcatctgctcgggcctggcctaaaatgcacacagtcaatggttatgtaaacaggtctctgccaggtctgattggatgccacaggaaatcagtctattggcatgtgattggaatgggcaccactcctgaagtgcactcaatattcctcgaaggtcacacatttcttgtgaggaaccatcgccaggcgtccttggaaatctcgccaataactttccttactgctcaaacactcttgatggaccttggacagtttctactgttttgtcatatctcttcccaccaacatgatggcatggaagcttatgtcaaagtagacagctgtccagaggaaccccaactacgaatgaaaaataatgaagaagcggaagactatgatgatgatcttactgattctgaaatggatgtggtcaggtttgatgatgacaactctccttcctttatccaaattcgctcagttgccaagaagcatcctaaaacttgggtacattacattgctgctgaagaggaggactgggactatgctcccttagtcctcgcccccgatgacagaagttataaaagtcaatatttgaacaatggccctcagcggattggtaggaagtacaaaaaagtccgatttatggcatacacagatgaaacctttaagactcgtgaagctattcagcatgaatcaggaatcttgggacctttactttatggggaagttggagacacactgttgattatatttaagaatcaagcaagcagaccatataacatctaccctcacggaatcactgatgtccgtcctttgtattcaaggagattaccaaaaggtgtaaaacatttgaaggattttccaattctgccaggagaaatattcaaatataaatggacagtgactgtagaagatgggccaactaaatcagatcctcggtgcctgacccgctattactctagtttcgttaatatggagagagatctagcttcaggactcattggccctctcctcatctgctacaaagaatctgtagatcaaagaggaaaccagataatgtcagacaagaggaatgtcatcctgttttctgtatttgatgagaaccgaagctggtacctcacagagaatatacaacgctttctccccaatccagctggagtgcagcttgaggatccagagttccaagcctccaacatcatgcacagcatcaatggctatgtttttgatagtttgcagttgtcagtttgtttgcatgaggtggcatactggtacattctaagcattggagcacagactgacttcctttctgtcttcttctctggatataccttcaaacacaaaatggtctatgaagacacactcaccctattcccattctcaggagaaactgtcttcatgtcgatggaaaacccaggtctatggattctggggtgccacaactcagactttcggaacagaggcatgaccgccttactgaaggtttctagttgtgacaagaacactggtgattattacgaggacagttatgaagatatttcagcatacttgctgagtaaaaacaatgccattgaaccaagaagcttctctcaaaacccaccagtcttgaaacgccatcaacgggaaataactcgtactactcttcagtcagatcaagaggaaattgactatgatgataccatatcagttgaaatgaagaaggaagattttgacatttatgatgaggatgaaaatcagagcccccgcagctttcaaaagaaaacacgacactattttattgctgcagtggagaggctctgggattatgggatgagtagctccccacatgttctaagaaacagggctcagagtggcagtgtccctcagttcaagaaagttgttttccaggaatttactgatggctcctttactcagcccttataccgtggagaactaaatgaacatttgggactcctggggccatatataagagcagaagttgaagataatatcatggtaactttcagaaatcaggcctctcgtccctattccttctattctagccttatttcttatgaggaagatcagaggcaaggagcagaacctagaaaaaactttgtcaagcctaatgaaaccaaaacttacttttggaaagtgcaacatcatatggcacccactaaagatgagtttgactgcaaagcctgggcttatttctctgatgttgacctggaaaaagatgtgcactcaggcctgattggaccccttctggtctgccacactaacacactgaaccctgctcatgggagacaagtgacagtacaggaatttgctctgtttttcaccatctttgatgagaccaaaagctggtacttcactgaaaatatggaaagaaactgcagggctccctgcaatatccagatggaagatcccacttttaaagagaattatcgcttccatgcaatcaatggctacataatggatacactacctggcttagtaatggctcaggatcaaaggattcgatggtatctgctcagcatgggcagcaatgaaaacatccattctattcatttcagtggacatgtgttcactgtacgaaaaaaagaggagtataaaatggcactgtacaatctctatccaggtgtttttgagacagtggaaatgttaccatccaaagctggaatttggcgggtggaatgccttattggcgagcatctacatgctgggatgagcacactttttctggtgtacagcaataagtgtcagactcccctgggaatggcttctggacacattagagattttcagattacagcttcaggacaatatggacagtgggccccaaagctggccagacttcattattccggatcaatcaatgcctggagcaccaaggagcccttttcttggatcaaggtggatctgttggcaccaatgattattcacggcatcaagacccagggtgcccgtcagaagttctccagcctctacatctctcagtttatcatcatgtatagtcttgatgggaagaagtggcagacttatcgaggaaattccactggaaccttaatggtcttctttggcaatgtggattcatctgggataaaacacaatatttttaaccctccaattattgctcgatacatccgtttgcacccaactcattatagcattcgcagcactcttcgcatggagttgatgggctgtgatttaaatagttgcagcatgccattgggaatggagagtaaagcaatatcagatgcacagattactgcttcatcctactttaccaatatgtttgccacctggtctccttcaaaagctcgacttcacctccaagggaggagtaatgcctggagacctcaggtgaataatccaaaagagtggctgcaagtggacttccagaagacaatgaaagtcacaggagtaactactcagggagtaaaatctctgcttaccagcatgtatgtgaaggagttcctcatctccagcagtcaagatggccatcagtggactctcttttttcagaatggcaaagtaaaggtttttcagggaaatcaagactccttcacacctgtggtgaactctctagacccaccgttactgactcgctaccttcgaattcacccccagagttgggtgcaccagattgccctgaggatggaggttctgggctgcgaggcacaggacctctacgacaaaactcacacatgcccaccgtgcccagctccagaactcctgggcggaccgtcagtcttcctcttccccccaaaacccaaggacaccctcatgatctcccggacccctgaggtcacatgcgtggtggtggacgtgagccacgaagaccctgaggtcaagttcaactggtacgtggacggcgtggaggtgcataatgccaagacaaagccgcgggaggagcagtacaacagcacgtaccgtgtggtcagcgtcctcaccgtcctgcaccaggactggctgaatggcaaggagtacaagtgcaaggtctccaacaaagccctcccagcccccatcgagaaaaccatctccaaagccaaagggcagccccgagaaccacaggtgtacaccctgcccccatcccgggatgagctgaccaagaaccaggtcagcctgacctgcctggtcaaaggcttctatcccagcgacatcgccgtggagtgggagagcaatgggcagccggagaacaactacaagaccacgcctcccgtgttggactccgacggctccttcttcctctacagcaagctcaccgtggacaagagcaggtggcagcaggggaacgtcttctcatgctccgtgatgcatgaggctctgcacaaccactacacgcagaagagcctctccctgtctccgggtaaa

SEQ ID NO: 2 - protein, 1684 aa, Artificial Sequence
  B-Domain Deleted FVIIIFc
MQIELSTCFFLCLLRFCFSATRRYYLGAVELSWDYMQSDLGELPVDARFPPRVPKSFPFNTSVVYKKTLFVEFTDHLFNIAKPRPPWMGLLGPTIQAEVYDTVVITLKNMASHPVSLHAVGVSYWKASEGAEYDDQTSQREKEDDKVFPGGSHTYVWQVLKENGPMASDPLCLTYSYLSHVDLVKDLNSGLIGALLVCREGSLAKEKTQTLHKFILLFAVFDEGKSWHSETKNSLMQDRDAASARAWPKMHTVNGYVNRSLPGLIGCHRKSVYWHVIGMGTTPEVHSIFLEGHTFLVRNHRQASLEISPITFLTAQTLLMDLGQFLLFCHISSHQHDGMEAYVKVDSCPEEPQLRMKNNEEAEDYDDDLTDSEMDVVRFDDDNSPSFIQIRSVAKKHPKTWVHYIAAEEEDWDYAPLVLAPDDRSYKSQYLNNGPQRIGRKYKKVRFMAYTDETFKTREAIQHESGILGPLLYGEVGDTLLIIFKNQASRPYNIYPHGITDVRPLYSRRLPKGVKHLKDFPILPGEIFKYKWTVTVEDGPTKSDPRCLTRYYSSFVNMERDLASGLIGPLLICYKESVDQRGNQIMSDKRNVILFSVFDENRSWYLTENIQRFLPNPAGVQLEDPEFQASNIMHSINGYVFDSLQLSVCLHEVAYWYILSIGAQTDFLSVFFSGYTFKHKMVYEDTLTLFPFSGETVFMSMENPGLWILGCHNSDFRNRGMTALLKVSSCDKNTGDYYEDSYEDISAYLLSKNNAIEPRSFSQNPPVLKRHQREITRTTLQSDQEEIDYDDTISVEMKKEDFDIYDEDENQSPRSFQKKTRHYFIAAVERLWDYGMSSSPHVLRNRAQSGSVPQFKKVVFQEFTDGSFTQPLYRGELNEHLGLLGPYIRAEVEDNIMVTFRNQASRPYSFYSSLISYEEDQRQGAEPRKNFVKPNETKTYFWKVQHHMAPTKDEFDCKAWAYFSDVDLEKDVHSGLIGPLLVCHTNTLNPAHGRQVTVQEFALFFTIFDETKSWYFTENMERNCRAPCNIQMEDPTFKENYRFHAINGYIMDTLPGLVMAQDQRIRWYLLSMGSNENIHSIHFSGHVFTVRKKEEYKMALYNLYPGVFETVEMLPSKAGIWRVECLIGEHLHAGMSTLFLVYSNKCQTPLGMASGHIRDFQITASGQYGQWAPKLARLHYSGSINAWSTKEPFSWIKVDLLAPMIIHGIKTQGARQKFSSLYISQFIIMYSLDGKKWQTYRGNSTGTLMVFFGNVDSSGIKHNIFNPPIIARYIRLHPTHYSIRSTLRMELMGCDLNSCSMPLGMESKAISDAQITASSYFTNMFATWSPSKARLHLQGRSNAWRPQVNNPKEWLQVDFQKTMKVTGVTTQGVKSLLTSMYVKEFLISSSQDGHQWTLFFQNGKVKVFQGNQDSFTPVVNSLDPPLLTRYLRIHPQSWVHQIALRMEVLGCEAQDLYDKTHTCPPCPAPELLGGPSVFLFPPKPKDTLMISRTPEVTCVVVDVSHEDPEVKFNWYVDGVEVHNAKTKPREEQYNSTYRVVSVLTVLHQDWLNGKEYKCKVSNKALPAPIEKTISKAKGQPREPQVYTLPPSRDELTKNQVSLTCLVKGFYPSDIAVEWESNGQPENNYKTTPPVLDSDGSFFLYSKLTVDKSRWQQGNVFSCSVMHEALHNHYTQKSLSLSPGK

SEQ ID NO: 3 - DNA, 741 bp, Artificial Sequence
  Fc Portion
atggagacagacacactcctgctatgggtactgctgctctgggttccaggttccactggtgacaaaactcacacatgcccaccgtgcccagcacctgaactcctgggaggaccgtcagtcttcctcttccccccaaaacccaaggacaccctcatgatctcccggacccctgaggtcacatgcgtggtggtggacgtgagccacgaagaccctgaggtcaagttcaactggtacgtggacggcgtggaggtgcataatgccaagacaaagccgcgggaggagcagtacaacagcacgtaccgtgtggtcagcgtcctcaccgtcctgcaccaggactggctgaatggcaaggagtacaagtgcaaggtctccaacaaagccctcccagcccccatcgagaaaaccatctccaaagccaaagggcagccccgagaaccacaggtgtacaccctgcccccatcccgcgatgagctgaccaagaaccaggtcagcctgacctgcctggtcaaaggcttctatcccagcgacatcgccgtggagtgggagagcaatgggcagccggagaacaactacaagaccacgcctcccgtgttggactccgacggctccttcttcctctacagcaagctcaccgtggacaagagcaggtggcagcaggggaacgtcttctcatgctccgtgatgcatgaggctctgcacaaccactacacgcagaagagcctctccctgtctccgggtaaa

SEQ ID NO: 4 - protein, 247 aa, Artificial Sequence
  Fc Portion
METDTLLLWVLLLWVPGSTGDKTHTCPPCPAPELLGGPSVFLFPPKPKDTLMISRTPEVTCVVVDVSHEDPEVKFNWYVDGVEVHNAKTKPREEQYNSTYRVVSVLTVLHQDWLNGKEYKCKVSNKALPAPIEKTISKAKGQPREPQVYTLPPSRDELTKNQVSLTCLVKGFYPSDIAVEWESNGQPENNYKTTPPVLDSDGSFFLYSKLTVDKSRWQQGNVFSCSVMHEALHNHYTQKSLSLSPGK

SEQ ID NO: 5 - DNA, 7734 bp, Artificial Sequence
  Full Length FVIIIFc
atgcaaatagagctctccacctgcttctttctgtgccttttgcgattctgctttagtgccaccagaagatactacctgggtgcagtggaactgtcatgggactatatgcaaagtgatctcggtgagctgcctgtggacgcaagatttcctcctagagtgccaaaatcttttccattcaacacctcagtcgtgtacaaaaagactctgtttgtagaattcacggatcaccttttcaacatcgctaagccaaggccaccctggatgggtctgctaggtcctaccatccaggctgaggtttatgatacagtggtcattacacttaagaacatggcttcccatcctgtcagtcttcatgctgttggtgtatcctactggaaagcttctgagggagctgaatatgatgatcagaccagtcaaagggagaaagaagatgataaagtcttccctggtggaagccatacatatgtctggcaggtcctgaaagagaatggtccaatggcctctgacccactgtgccttacctactcatatctttctcatgtggacctggtaaaagacttgaattcaggcctcattggagccctactagtatgtagagaagggagtctggccaaggaaaagacacagaccttgcacaaatttatactactttttgctgtatttgatgaagggaaaagttggcactcagaaacaaagaactccttgatgcaggatagggatgctgcatctgctcgggcctggcctaaaatgcacacagtcaatggttatgtaaacaggtctctgccaggtctgattggatgccacaggaaatcagtctattggcatgtgattggaatgggcaccactcctgaagtgcactcaatattcctcgaaggtcacacatttcttgtgaggaaccatcgccaggcgtccttggaaatctcgccaataactttccttactgctcaaacactcttgatggaccttggacagtttctactgttttgtcatatctcttcccaccaacatgatggcatggaagcttatgtcaaagtagacagctgtccagaggaaccccaactacgaatgaaaaataatgaagaagcggaagactatgatgatgatcttactgattctgaaatggatgtggtcaggtttgatgatgacaactctccttcctttatccaaattcgctcagttgccaagaagcatcctaaaacttgggtacattacattgctgctgaagaggaggactgggactatgctcccttagtcctcgcccccgatgacagaagttataaaagtcaatatttgaacaatggccctcagcggattggtaggaagtacaaaaaagtccgatttatggcatacacagatgaaacctttaagactcgtgaagctattcagcatgaatcaggaatcttgggacctttactttatggggaagttggagacacactgttgattatatttaagaatcaagcaagcagaccatataacatctaccctcacggaatcactgatgtccgtcctttgtattcaaggagattaccaaaaggtgtaaaacatttgaaggattttccaattctgccaggagaaatattcaaatataaatggacagtgactgtagaagatgggccaactaaatcagatcctcggtgcctgacccgctattactctagtttcgttaatatggagagagatctagcttcaggactcattggccctctcctcatctgctacaaagaatctgtagatcaaagaggaaaccagataatgtcagacaagaggaatgtcatcctgttttctgtatttgatgagaaccgaagctggtacctcacagagaatatacaacgctttctccccaatccagctggagtgcagcttgaggatccagagttccaagcctccaacatcatgcacagcatcaatggctatgtttttgatagtttgcagttgtcagtttgtttgcatgaggtggcatactggtacattctaagcattggagcacagactgacttcctttctgtcttcttctctggatataccttcaaacacaaaatggtctatgaagacacactcaccctattcccattctcaggagaaactgtcttcatgtcgatggaaaacccaggtctatggattctggggtgccacaactcagactttcggaacagaggcatgaccgccttactgaaggtttctagttgtgacaagaacactggtgattattacgaggacagttatgaagatatttcagcatacttgctgagtaaaaacaatgccattgaaccaagaagcttctcccagaattcaagacaccctagcactaggcaaaagcaatttaatgccaccacaattccagaaaatgacatagagaagactgacccttggtttgcacacagaacacctatgcctaaaatacaaaatgtctcctctagtgatttgttgatgctcttgcgacagagtcctactccacatgggctatccttatctgatctccaagaagccaaatatgagactttttctgatgatccatcacctggagcaatagacagtaataacagcctgtctgaaatgacacacttcaggccacagctccatcacagtggggacatggtatttacccctgagtcaggcctccaattaagattaaatgagaaactggggacaactgcagcaacagagttgaagaaacttgatttcaaagtttctagtacatcaaataatctgatttcaacaattccatcagacaatttggcagcaggtactgataatacaagttccttaggacccccaagtatgccagttcattatgatagtcaattagataccactctatttggcaaaaagtcatctccccttactgagtctggtggacctctgagcttgagtgaagaaaataatgattcaaagttgttagaatcaggtttaatgaatagccaagaaagttcatggggaaaaaatgtatcgtcaacagagagtggtaggttatttaaagggaaaagagctcatggacctgctttgttgactaaagataatgccttattcaaagttagcatctctttgttaaagacaaacaaaacttccaataattcagcaactaatagaaagactcacattgatggcccatcattattaattgagaatagtccatcagtctggcaaaatatattagaaagtgacactgagtttaaaaaagtgacacctttgattcatgacagaatgcttatggacaaaaatgctacagctttgaggctaaatcatatgtcaaataaaactacttcatcaaaaaacatggaaatggtccaacagaaaaaagagggccccattccaccagatgcacaaaatccagatatgtcgttctttaagatgctattcttgccagaatcagcaaggtggatacaaaggactcatggaaagaactctctgaactctgggcaaggccccagtccaaagcaattagtatccttaggaccagaaaaatctgtggaaggtcagaatttcttgtctgagaaaaacaaagtggtagtaggaaagggtgaatttacaaaggacgtaggactcaaagagatggtttttccaagcagcagaaacctatttcttactaacttggataatttacatgaaaataatacacacaatcaagaaaaaaaaattcaggaagaaatagaaaagaaggaaacattaatccaagagaatgtagttttgcctcagatacatacagtgactggcactaagaatttcatgaagaaccttttcttactgagcactaggcaaaatgtagaaggttcatatgacggggcatatgctccagtacttcaagattttaggtcattaaatgattcaacaaatagaacaaagaaacacacagctcatttctcaaaaaaaggggaggaagaaaacttggaaggcttgggaaatcaaaccaagcaaattgtagagaaatatgcatgcaccacaaggatatctcctaatacaagccagcagaattttgtcacgcaacgtagtaagagagctttgaaacaattcagactcccactagaagaaacagaacttgaaaaaaggataattgtggatgacacctcaacccagtggtccaaaaacatgaaacatttgaccccgagcaccctcacacagatagactacaatgagaaggagaaaggggccattactcagtctcccttatcagattgccttacgaggagtcatagcatccctcaagcaaatagatctccattacccattgcaaaggtatcatcatttccatctattagacctatatatctgaccagggtcctattccaagacaactcttctcatcttccagcagcatcttatagaaagaaagattctggggtccaagaaagcagtcatttcttacaaggagccaaaaaaaataacctttctttagccattctaaccttggagatgactggtgatcaaagagaggttggctccctggggacaagtgccacaaattcagtcacatacaagaaagttgagaacactgttctcccgaaaccagacttgcccaaaacatctggcaaagttgaattgcttccaaaagttcacatttatcagaaggacctattccctacggaaactagcaatgggtctcctggccatctggatctcgtggaagggagccttcttcagggaacagagggagcgattaagtggaatgaagcaaacagacctggaaaagttccctttctgagagtagcaacagaaagctctgcaaagactccctccaagctattggatcctcttgcttgggataaccactatggtactcagataccaaaagaagagtggaaatcccaagagaagtcaccagaaaaaacagcttttaagaaaaaggataccattttgtccctgaacgcttgtgaaagcaatcatgcaatagcagcaataaatgagggacaaaataagcccgaaatagaagtcacctgggcaaagcaaggtaggactgaaaggctgtgctctcaaaacccaccagtcttgaaacgccatcaacgggaaataactcgtactactcttcagtcagatcaagaggaaattgactatgatgataccatatcagttgaaatgaagaaggaagattttgacatttatgatgaggatgaaaatcagagcccccgcagctttcaaaagaaaacacgacactattttattgctgcagtggagaggctctgggattatgggatgagtagctccccacatgttctaagaaacagggctcagagtggcagtgtccctcagttcaagaaagttgttttccaggaatttactgatggctcctttactcagcccttataccgtggagaactaaatgaacatttgggactcctggggccatatataagagcagaagttgaagataatatcatggtaactttcagaaatcaggcctctcgtccctattccttctattctagccttatttcttatgaggaagatcagaggcaaggagcagaacctagaaaaaactttgtcaagcctaatgaaaccaaaacttacttttggaaagtgcaacatcatatggcacccactaaagatgagtttgactgcaaagcctgggcttatttctctgatgttgacctggaaaaagatgtgcactcaggcctgattggaccccttctggtctgccacactaacacactgaaccctgctcatgggagacaagtgacagtacaggaatttgctctgtttttcaccatctttgatgagaccaaaagctggtacttcactgaaaatatggaaagaaactgcagggctccctgcaatatccagatggaagatcccacttttaaagagaattatcgcttccatgcaatcaatggctacataatggatacactacctggcttagtaatggctcaggatcaaaggattcgatggtatctgctcagcatgggcagcaatgaaaacatccattctattcatttcagtggacatgtgttcactgtacgaaaaaaagaggagtataaaatggcactgtacaatctctatccaggtgtttttgagacagtggaaatgttaccatccaaagctggaatttggcgggtggaatgccttattggcgagcatctacatgctgggatgagcacactttttctggtgtacagcaataagtgtcagactcccctgggaatggcttctggacacattagagattttcagattacagcttcaggacaatatggacagtgggccccaaagctggccagacttcattattccggatcaatcaatgcctggagcaccaaggagcccttttcttggatcaaggtggatctgttggcaccaatgattattcacggcatcaagacccagggtgcccgtcagaagttctccagcctctacatctctcagtttatcatcatgtatagtcttgatgggaagaagtggcagacttatcgaggaaattccactggaaccttaatggtcttctttggcaatgtggattcatctgggataaaacacaatatttttaaccctccaattattgctcgatacatccgtttgcacccaactcattatagcattcgcagcactcttcgcatggagttgatgggctgtgatttaaatagttgcagcatgccattgggaatggagagtaaagcaatatcagatgcacagattactgcttcatcctactttaccaatatgtttgccacctggtctccttcaaaagctcgacttcacctccaagggaggagtaatgcctggagacctcaggtgaataatccaaaagagtggctgcaagtggacttccagaagacaatgaaagtcacaggagtaactactcagggagtaaaatctctgcttaccagcatgtatgtgaaggagttcctcatctccagcagtcaagatggccatcagtggactctcttttttcagaatggcaaagtaaaggtttttcagggaaatcaagactccttcacacctgtggtgaactctctagacccaccgttactgactcgctaccttcgaattcacccccagagttgggtgcaccagattgccctgaggatggaggttctgggctgcgaggcacaggacctctacgacaaaactcacacatgcccaccgtgcccagctccagaactcctgggcggaccgtcagtcttcctcttccccccaaaacccaaggacaccctcatgatctcccggacccctgaggtcacatgcgtggtggtggacgtgagccacgaagaccctgaggtcaagttcaactggtacgtggacggcgtggaggtgcataatgccaagacaaagccgcgggaggagcagtacaacagcacgtaccgtgtggtcagcgtcctcaccgtcctgcaccaggactggctgaatggcaaggagtacaagtgcaaggtctccaacaaagccctcccagcccccatcgagaaaaccatctccaaagccaaagggcagccccgagaaccacaggtgtacaccctgcccccatcccgggatgagctgaccaagaaccaggtcagcctgacctgcctggtcaaaggcttctatcccagcgacatcgccgtggagtgggagagcaatgggcagccggagaacaactacaagaccacgcctcccgtgttggactccgacggctccttcttcctctacagcaagctcaccgtggacaagagcaggtggcagcaggggaacgtcttctcatgctccgtgatgcatgaggctctgcacaaccactacacgcagaagagcctctccctgtctccgggtaaa

SEQ ID NO: 6 - protein, 2578 aa, Artificial Sequence
  Full Length FVIIIFc
MQIELSTCFFLCLLRFCFSATRRYYLGAVELSWDYMQSDLGELPVDARFPPRVPKSFPFNTSVVYKKTLFVEFTDHLFNIAKPRPPWMGLLGPTIQAEVYDTVVITLKNMASHPVSLHAVGVSYWKASEGAEYDDQTSQREKEDDKVFPGGSHTYVWQVLKENGPMASDPLCLTYSYLSHVDLVKDLNSGLIGALLVCREGSLAKEKTQTLHKFILLFAVFDEGKSWHSETKNSLMQDRDAASARAWPKMHTVNGYVNRSLPGLIGCHRKSVYWHVIGMGTTPEVHSIFLEGHTFLVRNHRQASLEISPITFLTAQTLLMDLGQFLLFCHISSHQHDGMEAYVKVDSCPEEPQLRMKNNEEAEDYDDDLTDSEMDVVRFDDDNSPSFIQIRSVAKKHPKTWVHYIAAEEEDWDYAPLVLAPDDRSYKSQYLNNGPQRIGRKYKKVRFMAYTDETFKTREAIQHESGILGPLLYGEVGDTLLIIFKNQASRPYNIYPHGITDVRPLYSRRLPKGVKHLKDFPILPGEIFKYKWTVTVEDGPTKSDPRCLTRYYSSFVNMERDLASGLIGPLLICYKESVDQRGNQIMSDKRNVILFSVFDENRSWYLTENIQRFLPNPAGVQLEDPEFQASNIMHSINGYVFDSLQLSVCLHEVAYWYILSIGAQTDFLSVFFSGYTFKHKMVYEDTLTLFPFSGETVFMSMENPGLWILGCHNSDFRNRGMTALLKVSSCDKNTGDYYEDSYEDISAYLLSKNNAIEPRSFSQNSRHPSTRQKQFNATTIPENDIEKTDPWFAHRTPMPKIQNVSSSDLLMLLRQSPTPHGLSLSDLQEAKYETFSDDPSPGAIDSNNSLSEMTHFRPQLHHSGDMVFTPESGLQLRLNEKLGTTAATELKKLDFKVSSTSNNLISTIPSDNLAAGTDNTSSLGPPSMPVHYDSQLDTTLFGKKSSPLTESGGPLSLSEENNDSKLLESGLMNSQESSWGKNVSSTESGRLFKGKRAHGPALLTKDNALFKVSISLLKTNKTSNNSATNRKTHIDGPSLLIENSPSVWQNILESDTEFKKVTPLIHDRMLMDKNATALRLNHMSNKTTSSKNMEMVQQKKEGPIPPDAQNPDMSFFKMLFLPESARWIQRTHGKNSLNSGQGPSPKQLVSLGPEKSVEGQNFLSEKNKVVVGKGEFTKDVGLKEMVFPSSRNLFLTNLDNLHENNTHNQEKKIQEEIEKKETLIQENVVLPQIHTVTGTKNFMKNLFLLSTRQNVEGSYDGAYAPVLQDFRSLNDSTNRTKKHTAHFSKKGEEENLEGLGNQTKQIVEKYACTTRISPNTSQQNFVTQRSKRALKQFRLPLEETELEKRIIVDDTSTQWSKNMKHLTPSTLTQIDYNEKEKGAITQSPLSDCLTRSHSIPQANRSPLPIAKVSSFPSIRPIYLTRVLFQDNSSHLPAASYRKKDSGVQESSHFLQGAKKNNLSLAILTLEMTGDQREVGSLGTSATNSVTYKKVENTVLPKPDLPKTSGKVELLPKVHIYQKDLFPTETSNGSPGHLDLVEGSLLQGTEGAIKWNEANRPGKVPFLRVATESSAKTPSKLLDPLAWDNHYGTQIPKEEWKSQEKSPEKTAFKKKDTILSLNACESNHAIAAINEGQNKPEIEVTWAKQGRTERLCSQNPPVLKRHQREITRTTLQSDQEEIDYDDTISVEMKKEDFDIYDEDENQSPRSFQKKTRHYFIAAVERLWDYGMSSSPHVLRNRAQSGSVPQFKKVVFQEFTDGSFTQPLYRGELNEHLGLLGPYIRAEVEDNIMVTFRNQASRPYSFYSSLISYEEDQRQGAEPRKNFVKPNETKTYFWKVQHHMAPTKDEFDCKAWAYFSDVDLEKDVHSGLIGPLLVCHTNTLNPAHGRQVTVQEFALFFTIFDETKSWYFTENMERNCRAPCNIQMEDPTFKENYRFHAINGYIMDTLPGLVMAQDQRIRWYLLSMGSNENIHSIHFSGHVFTVRKKEEYKMALYNLYPGVFETVEMLPSKAGIWRVECLIGEHLHAGMSTLFLVYSNKCQTPLGMASGHIRDFQITASGQYGQWAPKLARLHYSGSINAWSTKEPFSWIKVDLLAPMIIHGIKTQGARQKFSSLYISQFIIMYSLDGKKWQTYRGNSTGTLMVFFGNVDSSGIKHNIFNPPIIARYIRLHPTHYSIRSTLRMELMGCDLNSCSMPLGMESKAISDAQITASSYFTNMFATWSPSKARLHLQGRSNAWRPQVNNPKEWLQVDFQKTMKVTGVTTQGVKSLLTSMYVKEFLISSSQDGHQWTLFFQNGKVKVFQGNQDSFTPVVNSLDPPLLTRYLRIHPQSWVHQIALRMEVLGCEAQDLYDKTHTCPPCPAPELLGGPSVFLFPPKPKDTLMISRTPEVTCVVVDVSHEDPEVKFNWYVDGVEVHNAKTKPREEQYNSTYRVVSVLTVLHQDWLNGKEYKCKVSNKALPAPIEKTISKAKGQPREPQVYTLPPSRDELTKNQVSLTCLVKGFYPSDIAVEWESNGQPENNYKTTPPVLDSDGSFFLYSKLTVDKSRWQQGNVFSCSVMHEALHNHYTQKSLSLSPGK

SEQ ID NO: 7 - protein, 11 aa, Artificial Sequence
  Albumin-binding Peptide Core
DICLPRWGCLW

SEQ ID NO: 8 - protein, 32 aa, Artificial Sequence
  CTP peptide
DPRFQDSSSSKAPPPSLPSPSRLPGPSDTPIL

SEQ ID NO: 9 - protein, 28 aa, Artificial Sequence
  CTP peptide
SSSSKAPPPSLPSPSRLPGPSDTPILPQ

SEQ ID NO: 10 - protein, 20 aa, Artificial Sequence
  PAS peptide
ASPAAPAPASPAAPAPSAPA

SEQ ID NO: 11 - protein, 20 aa, Artificial Sequence
  PAS peptide
AAPASPAPAAPSAPAPAAPS

SEQ ID NO: 12 - protein, 20 aa, Artificial Sequence
  PAS peptide
APSSPSPSAPSSPSPASPSS

SEQ ID NO: 13 - protein, 19 aa, Artificial Sequence
  PAS peptide
APSSPSPSAPSSPSPASPS

SEQ ID NO: 14 - protein, 20 aa, Artificial Sequence
  PAS peptide
SSPSAPSPSSPASPSPSSPA

SEQ ID NO: 15 - protein, 24 aa, Artificial Sequence
  PAS peptide
AASPAAPSAPPAAASPAAPSAPPA

SEQ ID NO: 16 - protein, 20 aa, Artificial Sequence
  PAS peptide
ASAAAPAAASAAASAPSAAA

SEQ ID NO: 17 - protein, 21 aa, Artificial Sequence
  fragment of Factor VIII B domain
SFSQNSRHPSQNPPVLKRHQR

SEQ ID NO: 18 - protein, 6 aa, Artificial Sequence
  His tag
HHHHHH